European Patent Specification EP 3 820 882 B1, published April 2, 2025. Title: PEPTIDE COMPOUNDS AND THERAPEUTIC USES OF SAME. Applicant: Immunity Pharma Ltd. OVADIA, Eran BEN-SHIMON, Avi. The sequence listing filed with the application follows.

SEQUENCE LISTING (21 sequences)

SEQ ID NO: 1 - protein, 5 aa, Artificial sequence
  peptide
  MISC_FEATURE (1)..(2): X  is proline or an analogue or derivative thereof
  MISC_FEATURE (3)..(3): X  is   alanine, valine, leucine, cysteine, isoleucine, methionine or a derivative or analogue thereof
  MISC_FEATURE (4)..(4): X  is   alanine, valine, serine, proline or a derivative or analogue thereof
  MISC_FEATURE (5)..(5): X  is  any amino acid
XXXXX

SEQ ID NO: 2 - protein, 7 aa, Artificial sequence
  Stressin-1 amino acid sequence
LPPLPYP

SEQ ID NO: 3 - protein, 5 aa, Artificial sequence
  Synthetic Peptide
PPLPY

SEQ ID NO: 4 - protein, 7 aa, Artificial sequence
  Synthetic Peptide
LPPLAYP

SEQ ID NO: 5 - protein, 5 aa, Artificial sequence
  Synthetic Peptide
  misc_feature (1)..(1): Xaa can be any naturally occurring amino acid
  MISC_FEATURE (2)..(2): X2 is proline or an analogue or derivative thereof
  misc_feature (3)..(3): Xaa can be any naturally occurring amino acid
  MISC_FEATURE (4)..(4): X  is not proline
  misc_feature (5)..(5): Xaa can be any naturally occurring amino acid
XXXXX

SEQ ID NO: 6 - protein, 7 aa, Artificial sequence
  Synthetic Peptide
  misc_feature (1)..(1): Xaa can be any naturally occurring amino acid
  MISC_FEATURE (2)..(3): X is proline or an analogue or derivative thereof
  MISC_FEATURE (4)..(4): X is not proline
  misc_feature (5)..(6): Xaa can be any naturally occurring amino acid
  MISC_FEATURE (7)..(7): X is proline or an analogue or derivative thereof
XXXXXXX

SEQ ID NO: 7 - protein, 6 aa, Artificial sequence
  Synthetic Peptide
LPPLPY

SEQ ID NO: 8 - protein, 6 aa, Artificial sequence
  Synthetic Peptide
PPLPYP

SEQ ID NO: 9 - protein, 5 aa, Artificial sequence
  Synthetic Peptide
PLPYP

SEQ ID NO: 10 - protein, 3 aa, Artificial sequence
  Synthetic Peptide
PPL

SEQ ID NO: 11 - protein, 3 aa, Artificial sequence
  Synthetic Peptide
PLP

SEQ ID NO: 12 - protein, 3 aa, Artificial sequence
  Synthetic Peptide
PYP

SEQ ID NO: 13 - protein, 7 aa, Artificial sequence
  Synthetic Peptide
LPGLPYP

SEQ ID NO: 14 - protein, 7 aa, Artificial sequence
  Synthetic Peptide
LPPLGYP

SEQ ID NO: 15 - protein, 7 aa, Artificial sequence
  Synthetic Peptide
LAPLPYP

SEQ ID NO: 16 - protein, 7 aa, Artificial sequence
  Synthetic Peptide
LPALPYP

SEQ ID NO: 17 - protein, 6 aa, Artificial Sequence
  Synthetic Peptide
  MISC_FEATURE (1)..(1): X  is proline, or an analogue or derivative thereof
  MISC_FEATURE (2)..(2): X  is  proline, or an analogue or thereof
  MISC_FEATURE (3)..(3): X  is  eitherf alanine, valine, leucine, cysteine, isoleucine, methionine and a derivative or analogue thereof
  MISC_FEATURE (4)..(4): X  is  eitherf alanine, valine, serine and a derivative or analogue thereof
  misc_feature (5)..(5): Xaa can be any naturally occurring amino acid
  MISC_FEATURE (6)..(6): X  is  proline or an analogue or derivative thereof
XXXXXX

SEQ ID NO: 18 - protein, 6 aa, Artificial Sequence
  Synthetic Peptide
PPLAYP

SEQ ID NO: 19 - protein, 5 aa, Artificial Sequence
  Synthetic Peptide
  MOD_RES (5)..(5): AMIDATION
PPLPY

SEQ ID NO: 20 - protein, 6 aa, Artificial Sequence
  Synthetic Peptide
  MISC_FEATURE (1)..(1): may be D amino acid
  MISC_FEATURE (3)..(3): may be D amino acid
LPPLPY

SEQ ID NO: 21 - protein, 7 aa, Artificial Sequence
  Synthetic Peptide
  MISC_FEATURE (1)..(1): may be D amino acid
  MISC_FEATURE (3)..(3): may be D amino acid
  MISC_FEATURE (5)..(5): may be D amino acid
LPPLAYP